European Patent Specification EP 3 307 768 B1, published January 29, 2025. Title: SELECTIVE PYY COMPOUNDS AND USES THEREOF. Applicant: NOVO NORDISK A/S. The sequence listing filed with the application follows.

SEQUENCE LISTING (29 sequences)

SEQ ID NO: 1 - protein, 36 aa, HOMO SAPIENS
YPIKPEAPGEDASPEELNRYYASLRHYLNLVTRQRY

SEQ ID NO: 2 - protein, 34 aa, HOMO SAPIENS
IKPEAPGEDASPEELNRYYASLRHYLNLVTRQRY

SEQ ID NO: 3 - protein, 34 aa, ARTIFICIAL
  Artificial protein based on human PYY
  MISC_FEATURE (34)..(34): AMIDATION
IRPEKPGEDASPEELQRYYASLRHYYNWLTRQRY

SEQ ID NO: 4 - protein, 33 aa, ARTIFICIAL
  Artificial protein based on human PYY
  MISC_FEATURE (33)..(33): AMIDATION
RPEKPGEDASPEELQRYYASLRHYYNWLTRQRY

SEQ ID NO: 5 - protein, 33 aa, ARTIFICIAL
  Artificial protein based on human PYY
  MISC_FEATURE (33)..(33): AMIDATION
RPEKPPEDASPEELQRYYASLRHYYNWLTRQRY

SEQ ID NO: 6 - protein, 33 aa, ARTIFICIAL
  Artificial protein based on human PYY
  MISC_FEATURE (33)..(33): AMIDATION
RPEKPSEDASPEELQRYYASLRHYYNWLTRQRY

SEQ ID NO: 7 - protein, 33 aa, ARTIFICIAL
  Artificial protein based on human PYY
  MISC_FEATURE (33)..(33): AMIDATION
RPEKPTEDASPEELQRYYASLRHYYNWLTRQRY

SEQ ID NO: 8 - protein, 33 aa, ARTIFICIAL
  Artificial protein based on human PYY
  MISC_FEATURE (33)..(33): AMIDATION
RPEKPGEDATPEELQRYYASLRHYYNWLTRQRY

SEQ ID NO: 9 - protein, 33 aa, ARTIFICIAL
  Artificial protein based on human PYY
  MISC_FEATURE (33)..(33): AMIDATION
RPEKPGEDASPEELQRYYASARHYYNWLTRQRY

SEQ ID NO: 10 - protein, 33 aa, ARTIFICIAL
  Artificial protein based on human PYY
  MISC_FEATURE (33)..(33): AMIDATION
RPEKPGEDASPEELQRYYASIRHYYNWLTRQRY

SEQ ID NO: 11 - protein, 34 aa, ARTIFICIAL
  Artificial protein based on human PYY
  MISC_FEATURE (34)..(34): AMIDATION
ZRPEKPGEDASPEELQRYYASIRHYYNWLTRQRY

SEQ ID NO: 12 - protein, 34 aa, ARTIFICIAL
  Artificial protein based on human PYY
  MISC_FEATURE (34)..(34): AMIDATION
IRPEKPGEDASPEELQRYYISLRHYLNWLTRQRY

SEQ ID NO: 13 - protein, 33 aa, ARTIFICIAL
  Artificial protein based on human PYY
  MISC_FEATURE (33)..(33): AMIDATION
RPEKPGEDASPEELQRYYISLRHYLNWLTRQRY

SEQ ID NO: 14 - protein, 33 aa, ARTIFICIAL
  Artificial protein based on human PYY
  MISC_FEATURE (33)..(33): AMIDATION
RPEKPPEDASPEELQRYYISLRHYLNWLTRQRY

SEQ ID NO: 15 - protein, 33 aa, ARTIFICIAL
  Artificial protein based on human PYY
  MISC_FEATURE (33)..(33): AMIDATION
RPEKPGEDASPEELQRYYISLRHYYNWLTRQRY

SEQ ID NO: 16 - protein, 33 aa, ARTIFICIAL
  Artificial protein based on human PYY
  MISC_FEATURE (33)..(33): AMIDATION
RPEKPGEDASPEELQRYYISARHYYNWLTRQRY

SEQ ID NO: 17 - protein, 33 aa, ARTIFICIAL
  Artificial protein based on human PYY
  MISC_FEATURE (33)..(33): AMIDATION
RPEKPGEDASPEELQRYYQSLRHYYNWLTRQRY

SEQ ID NO: 18 - protein, 33 aa, ARTIFICIAL
  Artificial protein based on human PYY
  MISC_FEATURE (33)..(33): AMIDATION
RPEKPGEDASPEELQRYYVSLRHYYNWLTRQRY

SEQ ID NO: 19 - protein, 33 aa, ARTIFICIAL
  Artificial protein based on human PYY
  MISC_FEATURE (33)..(33): AMIDATION
RPEKPTEDASPEELQRYYQSLRHYYNWLTRQRY

SEQ ID NO: 20 - protein, 33 aa, ARTIFICIAL
  Artificial protein based on human PYY
  MISC_FEATURE (33)..(33): AMIDATION
RPEKPTEDASPEELQRYYVSLRHYYNWLTRQRY

SEQ ID NO: 21 - protein, 33 aa, ARTIFICIAL
  Artificial protein based on human PYY
  MISC_FEATURE (33)..(33): AMIDATION
RPEKPGEDATPEELQRYYQSLRHYYNWLTRQRY

SEQ ID NO: 22 - protein, 33 aa, ARTIFICIAL
  Artificial protein based on human PYY
  MISC_FEATURE (33)..(33): AMIDATION
RPEKPGEDATPEELQRYYVSLRHYYNWLTRQRY

SEQ ID NO: 23 - protein, 33 aa, Artificial Sequence
  Artificial protein based on human PYY
  MISC_FEATURE (33)..(33): Amidation
RPEAPGKDASPEELQRYYESLRHYYNWLTRQRY

SEQ ID NO: 24 - protein, 33 aa, Artificial Sequence
  Artificial protein based on human PYY
  MISC_FEATURE (33)..(33): Amidation
RPEAPGKDASPEELQRYYAELRHYYNWLTRQRY

SEQ ID NO: 25 - protein, 33 aa, Artificial Sequence
  Artificial protein based on human PYY
  MISC_FEATURE (33)..(33)
  MOD_RES (33)..(33): AMIDATION
RPEAPPKDASPEELQRYYESLRHYYNWLTRQRY

SEQ ID NO: 26 - protein, 33 aa, Artificial Sequence
  Artificial protein based on human PYY
  MOD_RES (33)..(33): AMIDATION
RPEAPPKDASPEELQRYYASLRHYYNWLTRQRY

SEQ ID NO: 27 - protein, 33 aa, Artificial Sequence
  Artificial protein based on human PYY
  MOD_RES (33)..(33): AMIDATION
RPEAPGKDASPEELQRYYASLRHYYNWLTRQRY

SEQ ID NO: 28 - protein, 33 aa, Artificial Sequence
  Artificial protein based on human PYY
  MOD_RES (33)..(33): AMIDATION
RPEAPGEDASPEELQRYYASLRHYYNWLTRQRY

SEQ ID NO: 29 - protein, 33 aa, Artificial Sequence
  Artificial protein based on human PYY
  MISC_FEATURE (33)..(33): AMIDATION
RPEAPGEDASPEELQRYYVSLRHYYNWLTRQRY